European Patent Specification EP 3 896 078 B1, published November 19, 2025. Title: ANTI-INFLAMMATORY PEPTIDES AND COMPOSITION COMPRISING THE SAME. Applicant: KAEL-GemVax Co., Ltd. GemVax AS KIM, Sangjae. The sequence listing filed with the application follows.

SEQUENCE LISTING (163 sequences)

SEQ ID NO: 1 - protein, 30 aa, Homo sapiens
ALFSVLNYERARRPGLLGASVLGLDDIHRA

SEQ ID NO: 2 - protein, 15 aa, Homo sapiens
SVLNYERARRPGLLG

SEQ ID NO: 3 - protein, 10 aa, Homo sapiens
GLLGASVLGL

SEQ ID NO: 4 - protein, 10 aa, Homo sapiens
ALLTSRLRFI

SEQ ID NO: 5 - protein, 9 aa, Homo sapiens
RPALLTSRL

SEQ ID NO: 6 - protein, 9 aa, Homo sapiens
RLTSRVKAL

SEQ ID NO: 7 - protein, 15 aa, Homo sapiens
RTFVLRVRAQDPPPE

SEQ ID NO: 8 - protein, 15 aa, Homo sapiens
RLTSRVKALFSVLNY

SEQ ID NO: 9 - protein, 15 aa, Homo sapiens
AERLTSRVKALFSVL

SEQ ID NO: 10 - protein, 9 aa, Homo sapiens
YERARRPGL

SEQ ID NO: 11 - protein, 9 aa, Homo sapiens
LLGASVLGL

SEQ ID NO: 12 - protein, 10 aa, Homo sapiens
VLGLDDIHRA

SEQ ID NO: 13 - protein, 10 aa, Homo sapiens
GASVLGLDDI

SEQ ID NO: 14 - protein, 10 aa, Homo sapiens
ALFSVLNYER

SEQ ID NO: 15 - protein, 10 aa, Homo sapiens
SVLNYERARR

SEQ ID NO: 16 - protein, 10 aa, Homo sapiens
SVLGLDDIHR

SEQ ID NO: 17 - protein, 10 aa, Homo sapiens
FSVLNYERAR

SEQ ID NO: 18 - protein, 10 aa, Homo sapiens
NYERARRPGL

SEQ ID NO: 19 - protein, 10 aa, Homo sapiens
YERARRPGLL

SEQ ID NO: 20 - protein, 10 aa, Homo sapiens
RPGLLGASVL

SEQ ID NO: 21 - protein, 9 aa, Homo sapiens
ERARRPGLL

SEQ ID NO: 22 - protein, 9 aa, Homo sapiens
VLGLDDIHR

SEQ ID NO: 23 - protein, 9 aa, Homo sapiens
SVLNYERAR

SEQ ID NO: 24 - protein, 9 aa, Homo sapiens
VLNYERARR

SEQ ID NO: 25 - protein, 9 aa, Homo sapiens
ARRPGLLGA

SEQ ID NO: 26 - protein, 9 aa, Homo sapiens
PGLLGASVL

SEQ ID NO: 27 - protein, 9 aa, Homo sapiens
RRPGLLGAS

SEQ ID NO: 28 - protein, 9 aa, Homo sapiens
ALFSVLNYE

SEQ ID NO: 29 - protein, 9 aa, Homo sapiens
GLLGASVLG

SEQ ID NO: 30 - protein, 9 aa, Homo sapiens
SVLGLDDIH

SEQ ID NO: 31 - protein, 8 aa, Homo sapiens
ERARRPGL

SEQ ID NO: 32 - protein, 8 aa, Homo sapiens
ARRPGLLG

SEQ ID NO: 33 - protein, 8 aa, Homo sapiens
GLLGASVL

SEQ ID NO: 34 - protein, 8 aa, Homo sapiens
RARRPGLL

SEQ ID NO: 35 - protein, 8 aa, Homo sapiens
LGASVLGL

SEQ ID NO: 36 - protein, 15 aa, Homo sapiens
VTETTFQKNRLFFYR

SEQ ID NO: 37 - protein, 15 aa, Homo sapiens
LFFYRKSVWSKLQSI

SEQ ID NO: 38 - protein, 15 aa, Homo sapiens
KLQSIGIRQHLKRVQ

SEQ ID NO: 39 - protein, 15 aa, Homo sapiens
EAEVRQHREARPALL

SEQ ID NO: 40 - protein, 15 aa, Homo sapiens
RPALLTSRLRFIPKP

SEQ ID NO: 41 - protein, 15 aa, Homo sapiens
FIPKPDGLRPIVNMD

SEQ ID NO: 42 - protein, 15 aa, Homo sapiens
RTFRREKRAERLTSR

SEQ ID NO: 43 - protein, 15 aa, Homo sapiens
LDDIHRAWRTFVLRV

SEQ ID NO: 44 - protein, 15 aa, Homo sapiens
FVLRVRAQDPPPELY

SEQ ID NO: 45 - protein, 15 aa, Homo sapiens
PQDRLTEVIASIIKP

SEQ ID NO: 46 - protein, 15 aa, Homo sapiens
KSVWSKLQSIGIRQH

SEQ ID NO: 47 - protein, 16 aa, Homo sapiens
LKRVQLRELSEAEVRQ

SEQ ID NO: 48 - protein, 20 aa, Homo sapiens
MPRAPRCRAVRSLLRSHYRE

SEQ ID NO: 49 - protein, 20 aa, Homo sapiens
VLPLATFVRRLGPQGWRLVQ

SEQ ID NO: 50 - protein, 20 aa, Homo sapiens
RGDPAAFRALVAQCLVCVPW

SEQ ID NO: 51 - protein, 20 aa, Homo sapiens
DARPPPAAPSFRQVSCLKEL

SEQ ID NO: 52 - protein, 20 aa, Homo sapiens
VARVLQRLCERGAKNVLAFG

SEQ ID NO: 53 - protein, 20 aa, Homo sapiens
FALLDGARGGPPEAFTTSVR

SEQ ID NO: 54 - protein, 20 aa, Homo sapiens
SYLPNTVTDALRGSGAWGLL

SEQ ID NO: 55 - protein, 20 aa, Homo sapiens
LRRVGDDVLVHLLARCALFV

SEQ ID NO: 56 - protein, 20 aa, Homo sapiens
LVAPSCAYQVCGPPLYQLGA

SEQ ID NO: 57 - protein, 20 aa, Homo sapiens
ATQARPPPHASGPRRRLGCE

SEQ ID NO: 58 - protein, 20 aa, Homo sapiens
RAWNHSVREAGVPLGLPAPG

SEQ ID NO: 59 - protein, 20 aa, Homo sapiens
ARRRGGSASRSLPLPKRPRR

SEQ ID NO: 60 - protein, 20 aa, Homo sapiens
GAAPEPERTPVGQGSWAHPG

SEQ ID NO: 61 - protein, 20 aa, Homo sapiens
RTRGPSDRGFCVVSPARPAE

SEQ ID NO: 62 - protein, 20 aa, Homo sapiens
EATSLEGALSGTRHSHPSVG

SEQ ID NO: 63 - protein, 20 aa, Homo sapiens
RQHHAGPPSTSRPPRPWDTP

SEQ ID NO: 64 - protein, 20 aa, Homo sapiens
CPPVYAETKHFLYSSGDKEQ

SEQ ID NO: 65 - protein, 20 aa, Homo sapiens
LRPSFLLSSLRPSLTGARRL

SEQ ID NO: 66 - protein, 20 aa, Homo sapiens
VETIFLGSRPWMPGTPRRLP

SEQ ID NO: 67 - protein, 20 aa, Homo sapiens
RLPQRYWQMRPLFLELLGNH

SEQ ID NO: 68 - protein, 20 aa, Homo sapiens
AQCPYGVLLKTHCPLRAAVT

SEQ ID NO: 69 - protein, 20 aa, Homo sapiens
PAAGVCAREKPQGSVAAPEE

SEQ ID NO: 70 - protein, 20 aa, Homo sapiens
EDTDPRRLVQLLRQHSSPWQ

SEQ ID NO: 71 - protein, 20 aa, Homo sapiens
VYGFVRACLRRLVPPGLWGS

SEQ ID NO: 72 - protein, 20 aa, Homo sapiens
RHNERRFLRNTKKFISLGKH

SEQ ID NO: 73 - protein, 20 aa, Homo sapiens
AKLSLQELTWKMSVRDCAWL

SEQ ID NO: 74 - protein, 20 aa, Homo sapiens
RRSPGVGCVPAAEHRLREEI

SEQ ID NO: 75 - protein, 20 aa, Homo sapiens
LAKFLHWLMSVYVVELLRSF

SEQ ID NO: 76 - protein, 20 aa, Homo sapiens
FYVTETTFQKNRLFFYRKSV

SEQ ID NO: 77 - protein, 20 aa, Homo sapiens
WSKLQSIGIRQHLKRVQLRE

SEQ ID NO: 78 - protein, 20 aa, Homo sapiens
LSEAEVRQHREARPALLTSR

SEQ ID NO: 79 - protein, 20 aa, Homo sapiens
LRFIPKPDGLRPIVNMDYVV

SEQ ID NO: 80 - protein, 20 aa, Homo sapiens
GARTFRREKRAERLTSRVKA

SEQ ID NO: 81 - protein, 20 aa, Homo sapiens
LFSVLNYERARRPGLLGASV

SEQ ID NO: 82 - protein, 20 aa, Homo sapiens
LGLDDIHRAWRTFVLRVRAQ

SEQ ID NO: 83 - protein, 20 aa, Homo sapiens
DPPPELYFVKVDVTGAYDTI

SEQ ID NO: 84 - protein, 20 aa, Homo sapiens
PQDRLTEVIASIIKPQNTYC

SEQ ID NO: 85 - protein, 20 aa, Homo sapiens
VRRYAVVQKAAHGHVRKAFK

SEQ ID NO: 86 - protein, 20 aa, Homo sapiens
SHVSTLTDLQPYMRQFVAHL

SEQ ID NO: 87 - protein, 20 aa, Homo sapiens
QETSPLRDAVVIEQSSSLNE

SEQ ID NO: 88 - protein, 20 aa, Homo sapiens
ASSGLFDVFLRFMCHHAVRI

SEQ ID NO: 89 - protein, 20 aa, Homo sapiens
RGKSYVQCQGIPQGSILSTL

SEQ ID NO: 90 - protein, 20 aa, Homo sapiens
LCSLCYGDMENKLFAGIRRD

SEQ ID NO: 91 - protein, 20 aa, Homo sapiens
GLLLRLVDDFLLVTPHLTHA

SEQ ID NO: 92 - protein, 20 aa, Homo sapiens
KTFLRTLVRGVPEYGCVVNL

SEQ ID NO: 93 - protein, 20 aa, Homo sapiens
RKTVVNFPVEDEALGGTAFV

SEQ ID NO: 94 - protein, 20 aa, Homo sapiens
QMPAHGLFPWCGLLLDTRTL

SEQ ID NO: 95 - protein, 20 aa, Homo sapiens
EVQSDYSSYARTSIRASLTF

SEQ ID NO: 96 - protein, 20 aa, Homo sapiens
NRGFKAGRNMRRKLFGVLRL

SEQ ID NO: 97 - protein, 20 aa, Homo sapiens
KCHSLFLDLQVNSLQTVCTN

SEQ ID NO: 98 - protein, 20 aa, Homo sapiens
IYKILLLQAYRFHACVLQLP

SEQ ID NO: 99 - protein, 20 aa, Homo sapiens
FHQQVWKNPTFFLRVISDTA

SEQ ID NO: 100 - protein, 20 aa, Homo sapiens
SLCYSILKAKNAGMSLGAKG

SEQ ID NO: 101 - protein, 20 aa, Homo sapiens
AAGPLPSEAVQWLCHQAFLL

SEQ ID NO: 102 - protein, 20 aa, Homo sapiens
KLTRHRVTYVPLLGSLRTAQ

SEQ ID NO: 103 - protein, 20 aa, Homo sapiens
TQLSRKLPGTTLTALEAAAN

SEQ ID NO: 104 - protein, 12 aa, Homo sapiens
PALPSDFKTILD

SEQ ID NO: 105 - protein, 10 aa, Homo sapiens
MPRAPRCRAV

SEQ ID NO: 106 - protein, 20 aa, Homo sapiens
RSLLRSHYREVLPLATFVRR

SEQ ID NO: 107 - protein, 20 aa, Homo sapiens
LGPQGWRLVQRGDPAAFRAL

SEQ ID NO: 108 - protein, 20 aa, Homo sapiens
VAQCLVCVPWDARPPPAAPS

SEQ ID NO: 109 - protein, 20 aa, Homo sapiens
FRQVSCLKELVARVLQRLCE

SEQ ID NO: 110 - protein, 20 aa, Homo sapiens
RGAKNVLAFGFALLDGARGG

SEQ ID NO: 111 - protein, 20 aa, Homo sapiens
PPEAFTTSVRSYLPNTVTDA

SEQ ID NO: 112 - protein, 20 aa, Homo sapiens
LRGSGAWGLLLRRVGDDVLV

SEQ ID NO: 113 - protein, 20 aa, Homo sapiens
HLLARCALFVLVAPSCAYQV

SEQ ID NO: 114 - protein, 20 aa, Homo sapiens
CGPPLYQLGAATQARPPPHA

SEQ ID NO: 115 - protein, 20 aa, Homo sapiens
SGPRRRLGCERAWNHSVREA

SEQ ID NO: 116 - protein, 20 aa, Homo sapiens
GVPLGLPAPGARRRGGSASR

SEQ ID NO: 117 - protein, 20 aa, Homo sapiens
SLPLPKRPRRGAAPEPERTP

SEQ ID NO: 118 - protein, 20 aa, Homo sapiens
VGQGSWAHPGRTRGPSDRGF

SEQ ID NO: 119 - protein, 20 aa, Homo sapiens
CVVSPARPAEEATSLEGALS

SEQ ID NO: 120 - protein, 20 aa, Homo sapiens
GTRHSHPSVGRQHHAGPPST

SEQ ID NO: 121 - protein, 20 aa, Homo sapiens
SRPPRPWDTPCPPVYAETKH

SEQ ID NO: 122 - protein, 20 aa, Homo sapiens
FLYSSGDKEQLRPSFLLSSL

SEQ ID NO: 123 - protein, 20 aa, Homo sapiens
RPSLTGARRLVETIFLGSRP

SEQ ID NO: 124 - protein, 20 aa, Homo sapiens
WMPGTPRRLPRLPQRYWQMR

SEQ ID NO: 125 - protein, 20 aa, Homo sapiens
PLFLELLGNHAQCPYGVLLK

SEQ ID NO: 126 - protein, 20 aa, Homo sapiens
THCPLRAAVTPAAGVCAREK

SEQ ID NO: 127 - protein, 20 aa, Homo sapiens
PQGSVAAPEEEDTDPRRLVQ

SEQ ID NO: 128 - protein, 20 aa, Homo sapiens
LLRQHSSPWQVYGFVRACLR

SEQ ID NO: 129 - protein, 20 aa, Homo sapiens
RLVPPGLWGSRHNERRFLRN

SEQ ID NO: 130 - protein, 20 aa, Homo sapiens
TKKFISLGKHAKLSLQELTW

SEQ ID NO: 131 - protein, 20 aa, Homo sapiens
KMSVRDCAWLRRSPGVGCVP

SEQ ID NO: 132 - protein, 20 aa, Homo sapiens
AAEHRLREEILAKFLHWLMS

SEQ ID NO: 133 - protein, 20 aa, Homo sapiens
VYVVELLRSFFYVTETTFQK

SEQ ID NO: 134 - protein, 20 aa, Homo sapiens
NRLFFYRKSVWSKLQSIGIR

SEQ ID NO: 135 - protein, 20 aa, Homo sapiens
QHLKRVQLRELSEAEVRQHR

SEQ ID NO: 136 - protein, 20 aa, Homo sapiens
EARPALLTSRLRFIPKPDGL

SEQ ID NO: 137 - protein, 20 aa, Homo sapiens
RPIVNMDYVVGARTFRREKR

SEQ ID NO: 138 - protein, 20 aa, Homo sapiens
AERLTSRVKALFSVLNYERA

SEQ ID NO: 139 - protein, 20 aa, Homo sapiens
RRPGLLGASVLGLDDIHRAW

SEQ ID NO: 140 - protein, 20 aa, Homo sapiens
RTFVLRVRAQDPPPELYFVK

SEQ ID NO: 141 - protein, 20 aa, Homo sapiens
VDVTGAYDTIPQDRLTEVIA

SEQ ID NO: 142 - protein, 20 aa, Homo sapiens
SIIKPQNTYCVRRYAVVQKA

SEQ ID NO: 143 - protein, 20 aa, Homo sapiens
AHGHVRKAFKSHVSTLTDLQ

SEQ ID NO: 144 - protein, 20 aa, Homo sapiens
PYMRQFVAHLQETSPLRDAV

SEQ ID NO: 145 - protein, 20 aa, Homo sapiens
VIEQSSSLNEASSGLFDVFL

SEQ ID NO: 146 - protein, 20 aa, Homo sapiens
RFMCHHAVRIRGKSYVQCQG

SEQ ID NO: 147 - protein, 20 aa, Homo sapiens
IPQGSILSTLLCSLCYGDME

SEQ ID NO: 148 - protein, 20 aa, Homo sapiens
NKLFAGIRRDGLLLRLVDDF

SEQ ID NO: 149 - protein, 20 aa, Homo sapiens
LLVTPHLTHAKTFLRTLVRG

SEQ ID NO: 150 - protein, 20 aa, Homo sapiens
VPEYGCVVNLRKTVVNFPVE

SEQ ID NO: 151 - protein, 20 aa, Homo sapiens
DEALGGTAFVQMPAHGLFPW

SEQ ID NO: 152 - protein, 20 aa, Homo sapiens
CGLLLDTRTLEVQSDYSSYA

SEQ ID NO: 153 - protein, 20 aa, Homo sapiens
RTSIRASLTFNRGFKAGRNM

SEQ ID NO: 154 - protein, 20 aa, Homo sapiens
RRKLFGVLRLKCHSLFLDLQ

SEQ ID NO: 155 - protein, 20 aa, Homo sapiens
VNSLQTVCTNIYKILLLQAY

SEQ ID NO: 156 - protein, 20 aa, Homo sapiens
RFHACVLQLPFHQQVWKNPT

SEQ ID NO: 157 - protein, 20 aa, Homo sapiens
FFLRVISDTASLCYSILKAK

SEQ ID NO: 158 - protein, 20 aa, Homo sapiens
NAGMSLGAKGAAGPLPSEAV

SEQ ID NO: 159 - protein, 20 aa, Homo sapiens
QWLCHQAFLLKLTRHRVTYV

SEQ ID NO: 160 - protein, 20 aa, Homo sapiens
PLLGSLRTAQTQLSRKLPGT

SEQ ID NO: 161 - protein, 22 aa, Homo sapiens
TLTALEAAANPALPSDFKTILD

SEQ ID NO: 162 - protein, 1132 aa, Homo sapiens
MPRAPRCRAVRSLLRSHYREVLPLATFVRRLGPQGWRLVQRGDPAAFRALVAQCLVCVPWDARPPPAAPSFRQVSCLKELVARVLQRLCERGAKNVLAFGFALLDGARGGPPEAFTTSVRSYLPNTVTDALRGSGAWGLLLRRVGDDVLVHLLARCALFVLVAPSCAYQVCGPPLYQLGAATQARPPPHASGPRRRLGCERAWNHSVREAGVPLGLPAPGARRRGGSASRSLPLPKRPRRGAAPEPERTPVGQGSWAHPGRTRGPSDRGFCVVSPARPAEEATSLEGALSGTRHSHPSVGRQHHAGPPSTSRPPRPWDTPCPPVYAETKHFLYSSGDKEQLRPSFLLSSLRPSLTGARRLVETIFLGSRPWMPGTPRRLPRLPQRYWQMRPLFLELLGNHAQCPYGVLLKTHCPLRAAVTPAAGVCAREKPQGSVAAPEEEDTDPRRLVQLLRQHSSPWQVYGFVRACLRRLVPPGLWGSRHNERRFLRNTKKFISLGKHAKLSLQELTWKMSVRDCAWLRRSPGVGCVPAAEHRLREEILAKFLHWLMSVYVVELLRSFFYVTETTFQKNRLFFYRKSVWSKLQSIGIRQHLKRVQLRELSEAEVRQHREARPALLTSRLRFIPKPDGLRPIVNMDYVVGARTFRREKRAERLTSRVKALFSVLNYERARRPGLLGASVLGLDDIHRAWRTFVLRVRAQDPPPELYFVKVDVTGAYDTIPQDRLTEVIASIIKPQNTYCVRRYAVVQKAAHGHVRKAFKSHVSTLTDLQPYMRQFVAHLQETSPLRDAVVIEQSSSLNEASSGLFDVFLRFMCHHAVRIRGKSYVQCQGIPQGSILSTLLCSLCYGDMENKLFAGIRRDGLLLRLVDDFLLVTPHLTHAKTFLRTLVRGVPEYGCVVNLRKTVVNFPVEDEALGGTAFVQMPAHGLFPWCGLLLDTRTLEVQSDYSSYARTSIRASLTFNRGFKAGRNMRRKLFGVLRLKCHSLFLDLQVNSLQTVCTNIYKILLLQAYRFHACVLQLPFHQQVWKNPTFFLRVISDTASLCYSILKAKNAGMSLGAKGAAGPLPSEAVQWLCHQAFLLKLTRHRVTYVPLLGSLRTAQTQLSRKLPGTTLTALEAAANPALPSDFKTILD

SEQ ID NO: 163 - protein, 16 aa, Homo sapiens
EARPALLTSRLRFIPK